European Patent Application EP 4 737 564 A1, published May 6, 2026. Title: 一种糖基转移酶UGTSL2突变体、糖基转移酶突变体及其合成莱鲍迪苷M2的方法. Applicant: 东台市浩瑞生物科技有限公司. The sequence listing filed with the application follows.

SEQUENCE LISTING (69 sequences)

SEQ ID NO: 1 - protein, 442 aa, synthetic construct
MATNLRVLMFPWLAYGHISPFLNIAKQLADRGFLIYLCSTRINLESIIKKIPEKYADSIHLIELQLPELPELPPHYHTTNGLPPHLNPTLHKALKMSKPNFSRILQNLKPDLLIYDVLQPWAEHVANEQNIPAGKLLTSCAAVFSYFFSFRKNPGVEFPFPAIHLPEVEKVKIREILAKEPEEGGRLDEGNKQMMLMCTSRTIEAKYIDYCTELCNWKVVPVGPPFQDLITNDADNKELIDWLGTKHENSTVFVSFGSEYFLSKEDMEEVAFALELSNVNFIWVARFPKGEERNLEDALPKGFLERIGERGRVLDKFAPQPRILNHPSTGGFISHCGWNSAMESIDFGVPIIAMPIHNDQPINAKLMVELGVAVEIVRDDDGKIHRGEIAETLKSVVTGETGEILRAKVREISKNLKSIRDEEMDAVAEELIQLCRNSNKSK

SEQ ID NO: 2 - DNA, 1326 bp, synthetic construct
  source 1..1326: mol_type = other DNA
atggcgaccaacctgcgtgtgctgatgttcccgtggctggcgtacggtcacatcagcccgtttctgaacattgcgaaacagctggcggatcgtggcttcctgatctacctgtgcagcacccgtattaacctggagagcatcattaagaaaatcccggaaaagtatgcggacagcatccacctgattgagctgcaactgccggagctgccggaactgccgccgcactatcacaccaccaacggtctgccgccgcacctgaacccgaccctgcacaaggcgctgaaaatgagcaagccgaactttagccgtatcctgcagaacctgaaaccggatctgctgatttacgacgtgctgcagccgtgggcggagcacgttgcgaacgaacaaaacattccggcgggtaaactgctgaccagctgcgcggcggtgttcagctatttctttagctttcgtaagaacccgggcgttgagttcccgtttccggcgatccacctgccggaagtggaaaaggttaaaatccgtgagattctggcgaaagaaccggaggaaggtggccgtctggatgagggtaacaagcagatgatgctgatgtgcaccagccgtaccatcgaggcgaaatacattgactattgcaccgaactgtgcaactggaaggtggttccggtgggtccgccgttccaagatctgatcaccaacgatgcggacaacaaagagctgattgactggctgggtaccaagcacgaaaacagcaccgtgttcgttagctttggcagcgagtacttcctgagcaaagaagatatggaggaagttgcgtttgcgctggagctgagcaacgtgaacttcatctgggttgcgcgttttccgaaaggcgaggaacgtaacctggaagatgcgctgccgaagggcttcctggagcgtattggtgaacgtggccgtgtgctggacaagtttgcgccgcagccgcgtatcctgaaccacccgagcaccggtggcttcattagccactgcggttggaacagcgcgatggagagcatcgattttggcgttccgatcattgcgatgccgatccacaacgaccaaccgattaacgcgaaactgatggtggagctgggtgtggcggttgaaatcgttcgtgacgatgacggtaaaatccaccgtggcgagattgcggaaaccctgaagagcgtggttaccggcgagaccggcgaaattctgcgtgcgaaagtgcgtgaaatcagcaaaaacctgaagagcattcgtgatgaggaaatggacgcggttgcggaggaactgatccaactgtgccgtaacagcaacaagagcaaa

SEQ ID NO: 3 - protein, 442 aa, synthetic construct
MATNLRVLMFPWLAYGHISPFLEIAKQLADRGFLIYLCSTPINLESIIKKIPEKYADSIHLIELQLPELPELPPHYHTTNGLPPHLNPTLKKALDMSKPNFSRILQNLKPDLLIYDVLQPWAPEVANEQNIPAGKFLTSCAAVFSYFFSFFKNPGVEFPFPAIHLPEYEKVKIREILAKEPEEGGRLDEGNKQMMLMKTSREIEAKYIDYCTELCNPKVVPVGPLVQDLITNDADNKELIDWLGTKHENSTVFVSFGSEYFLSKEDMEEVAFALELSNVNFIWVVRFPKGEERNLEDALPKGFLERIGERGRVLDKFAPQPRILNHPSTGGFVSHCGWNSAMESIDFGVPIIAMPIHFDQPINAKLMVELGVAVEIVRDDDGKIHRGEIAEVLKSVVTGETGEILRAKVREISKNLKSKRDEEMDAVAEELIQLCRNSNKSK

SEQ ID NO: 4 - DNA, 1326 bp, synthetic construct
  source 1..1326: mol_type = other DNA
atggcgaccaacctgcgtgtgctgatgttcccgtggctggcgtacggtcacatcagcccgtttctggaaattgcgaaacagctggcggatcgtggcttcctgatctacctgtgcagcaccccgattaacctggagagcatcattaagaaaatcccggaaaagtatgcggacagcatccacctgattgagctgcaactgccggagctgccggaactgccgccgcactatcacaccaccaacggtctgccgccgcacctgaacccgaccctgaaaaaggcgctggatatgagcaagccgaactttagccgtatcctgcagaacctgaaaccggatctgctgatttacgacgtgctgcagccgtgggcgccggaagttgcgaacgaacaaaacattccggcgggtaaatttctgaccagctgcgcggcggtgttcagctatttctttagcttttttaagaacccgggcgttgagttcccgtttccggcgatccacctgccggaatatgaaaaggttaaaatccgtgagattctggcgaaagaaccggaggaaggtggccgtctggatgagggtaacaagcagatgatgctgatgaaaaccagccgtgaaatcgaggcgaaatacattgactattgcaccgaactgtgcaacaaaaaggtggttccggtgggtccgctggttcaagatctgatcaccaacgatgcggacaacaaagagctgattgactggctgggtaccaagcacgaaaacagcaccgtgttcgttagctttggcagcgagtacttcctgagcaaagaagatatggaggaagttgcgtttgcgctggagctgagcaacgtgaacttcatctgggttgttcgttttccgaaaggcgaggaacgtaacctggaagatgcgctgccgaagggcttcctggagcgtattggtgaacgtggccgtgtgctggacaagtttgcgccgcagccgcgtatcctgaaccacccgagcaccggtggcttcgttagccactgcggttggaacagcgcgatggagagcatcgattttggcgttccgatcattgcgatgccgatccacttcgaccaaccgattaacgcgaaactgatggtggagctgggtgtggcggttgaaatcgttcgtgacgatgacggtaaaatccaccgtggcgagattgcggaagttctgaagagcgtggttaccggcgagaccggcgaaattctgcgtgcgaaagtgcgtgaaatcagcaaaaacctgaagagcaaacgtgatgaggaaatggacgcggttgcggaggaactgatccaactgtgccgtaacagcaacaagagcaaa

SEQ ID NO: 5 - protein, 454 aa, synthetic construct
MDTEHTKLKVFLFPWLAYGHISPFLELAKKLSDRGFLIELCSTPINLSFIKKRIPQSYSSTIQLVELILPELPQLPPHYHTTNGLPPHLNSTLHKALKLAKPNLFTILKTRKPDLIIYDVMQPWTFGVASSLNIPSARFFTSGAAMCSYFVHLYKNPEVEYPFPALHLYDYEIERARKLVQRNDKENENKDDQPEEEMPPQEGIMLISTSRELEGKYMDYLAEIIETRIFPIGTLVQDPVASGDENMNIMQWLDSKKELSTVFVSFGSEYFLTKEEREEIALGLELSQVNFIWVVRFPKGEKQNLEEALPQGFLERVGDRGMIVEWAPQAKILTHSSIGGFVSHCGWNSISESIEFGVPIIAIPMQLDQPMNAKLLVEIGVALEVVRDDNGSLHREEIASVIKDVTSGESSETMRCKVRNLGKNLRTKSVEDMDATVEELRELVGESRSKNGSF

SEQ ID NO: 6 - DNA, 1365 bp, synthetic construct
  source 1..1365: mol_type = other DNA
atggatactgaacacacaaaactaaaggttttcttgttcccgtggctggcgtatggtcatatttccccgtttttggagttggcgaagaaattgtctgatcgtggtttcctgatcgaactgtgttcgactccgatcaaccttagcttcatcaagaaacgtattccgcaaagctacagcagcacgatccagctggtggagctgatcctgccggagcttccgcaactgccaccgcattaccataccaccaacggtctgccgcctcacctgaacagcacgctgcacaaagcgttgaagcttgctaagccgaatttgttcaccattctgaaaaccagaaagccggatctgatcatctacgacgttatgcaaccttggacctttggcgtcgctagttcgctcaacatcccgagcgcacgcttctttacctcgggcgcggcaatgtgcagctatttcgttcatctctacaaaaaccctgaagttgagtacccgtttccggcacttcacctgtacgactacgaaatcgagcgtgcacgtaaactggtgcagcgtaacgataaagagaatgaaaacaaagacgaccagccagaagaagagatgccgcctcaagaaggtattatgctgattagcacgagccgtgagttggagggcaaatatatggactatttggctgaaatcatcgaaactcgcatttttccgatcggcactctggtacaggatccggttgccagcggtgacgagaacatgaatattatgcagtggctggacagcaaaaaggaattatctacggtttttgtgtccttcggctctgaatatttcttaaccaaagaggaacgtgaagagatagcgctgggtctggagttgagccaggttaattttatctgggttgttcgtttcccgaaaggcgaaaaacagaatctggaagaggcgctgccacaaggttttttggagcgcgtgggtgaccgcggtatgattgtggagtgggcaccgcaagcgaagatcctgacccacagctccattggcggcttcgtgagccactgcggttggaacagcatctcagaatctattgagtttggcgttccgattattgcgattccgatgcagctggaccaaccgatgaacgccaagttgctggtagagattggtgtggccctggaggtcgtgcgtgatgataatggctccctgcaccgtgaagagatcgcctccgtgattaaggacgtgacctctggggagagcagcgagaccatgcgttgcaaggtgcgcaacctgggtaagaacctgcgcaccaagagcgttgaagatatggatgcgaccgtcgaggaactgcgtgagctggtcggtgaatctagatccaagaacggcagcttttaa

SEQ ID NO: 7 - protein, 809 aa, synthetic construct
MANPKLTRVLSTRDRVQDTLSAHRNELVALLSRYVDQGKGILQPHNLIDELESVIGDDETKKSLSDGPFGEILKSAMEAIVVPPFVALAVRPRPGVWEYVRVNVFELSVEQLTVSEYLRFKEELVDGPNSDPFCLELDFEPFNANVPRPSRSSSIGNGVQFLNRHLSSVMFRNKDCLEPLLDFLRVHKYKGHPLMLNDRIQSISRLQIQLSKAEDHISKLSQETPFSEFEYALQGMGFEKGWGDTAGRVLEMMHLLSDILQAPDPSSLEKFLGMVPMVFNVVILSPHGYFGQANVLGLPDTGGQVVYILDQVRALETEMLLRIKRQGLDISPSILIVTRLIPDAKGTTCNQRLERVSGTEHTHILRVPFRSEKGILRKWISRFDVWPYLENYAQDAASEIVGELQGVPDFIIGNYSDGNLVASLMAHRMGVTQCTIAHALEKTKYPDSDIYWKDFDNKYHFSCQFTADLIAMNNADFIITSTYQEIAGTKNTVGQYESHGAFTLPGLYRVVHGIDVFDPKFNIVSPGADMTIYFPYSEETRRLTALHGSIEEMLYSPDQTDEHVGTLSDRSKPILFSMARLDKVKNISGLVEMYSKNTKLRELVNLVVIAGNIDVNKSKDREEIVEIEKMHNLMKNYKLDGQFRWITAQTNRARNGELYRYIADTRGAFAQPAFYEAFGLTVVEAMTCGLPTFATCHGGPAEIIEHGLSGFHIDPYHPEQAGNIMADFFERCKEDPNHWKKVSDAGLQRIYERYTWKIYSERLMTLAGVYGFWKYVSKLERRETRRYLEMFYILKFRDLVKTVPSTADD

SEQ ID NO: 8 - DNA, 2904 bp, synthetic construct
  source 1..2904: mol_type = other DNA
acgtcacttgtagcgaaaacagtatcaagaaaaagagaagatcaaacacgtcttcttttctctctctctctttgtcgcctaaaattccagaatcactctgctttttacccttttaatcaatgatttttccttttagtagcaatcgttggtgattcgaaaaaccaaacttttctcggactaggattctagggttttagtgatcatctgaatattcatggcaaaccctaagctcactagggttctaagcacaagggatcgcgtgcaagacacgctttccgctcaccgcaacgaactcgttgctcttctctccaggtatgtggatcaggggaaagggattcttcaaccacataacttaattgacgaactcgaatctgttatcggagacgatgaaacaaagaagagtctctctgatggtccttttggagagatccttaaatcagcaatggaagctatagttgtaccaccttttgttgcgttagccgttagaccaagacctggtgtttgggaatatgttcgtgttaatgtcttcgagctaagtgttgaacaattaacagtctctgagtatcttcgtttcaaagaagaactcgttgatggacctaatagtgaccctttttgtcttgagcttgatttcgagccctttaacgcaaacgtgccacgtccttctcgttcgtcttcgattggtaatggagttcagtttctgaatcgtcacttgtcttctgttatgttccgtaacaaagattgcttggagcctctgcttgatttccttagagttcataagtacaaaggtcatccgttgatgttgaatgatcggattcaaagcatatctaggcttcaaatccagcttagtaaagcagaagatcatatctctaagctttcacaagaaactccgttctcggaattcgaatacgcgttgcaaggaatgggttttgagaaaggatggggagataccgcagggagagttcttgaaatgatgcatcttctctctgatattcttcaagctcctgatccttcgtccttggagaagtttcttgggatggtaccaatggttttcaacgttgtgatcttatctccacatggatatttcgggcaagccaatgttttaggcttacctgacactggtggacaagttgtctatattcttgaccaagtccgtgcccttgagactgaaatgctgttgagaataaagagacaggggttggatatatcacctagtattcttattgtaactaggttgataccggatgctaaaggaactacgtgtaaccagcggttagagagagtcagcggaacagagcatactcatattctccgggttccttttaggtctgagaaaggaatcctccgtaagtggatttcaagattcgacgtatggccttatctagagaactatgctcaggatgcagcaagcgagattgtcggtgaattgcaaggcgtaccggactttatcatcggtaactatagtgacggaaaccttgttgcatcgttaatggcacatagaatgggtgttacacaatgtactattgcacatgctttggagaaaaccaagtatccagattcagacatttactggaaagacttcgacaacaagtatcatttctcttgtcaattcacagctgatcttatcgcaatgaacaacgcagatttcatcatcacaagcacttaccaagaaatcgcaggaacgaagaacaccgtcggtcaatatgaaagccacggggcttttacgctcccgggactatatagagtagtacacggcatcgatgtgtttgatccgaagttcaacatagtctcgcccggtgcagacatgaccatatatttcccgtattccgaagaaactaggagacttacagctttacatggttcaatagaggaaatgctctatagccctgaccagactgatgagcatgtcggtacactgagtgatcgatcaaagccaatactcttctctatggcgaggctcgacaaagtgaagaacatctccggtttagttgagatgtatagtaagaacacaaagttgagggagctggttaatctggttgtaatagctggtaacattgatgtgaacaagtccaaagatagagaagaaatcgtagagattgagaaaatgcataaccttatgaagaattacaagcttgatggacagtttcgttggataactgctcagactaaccgagctcgaaatggtgagctttaccgctacatcgcggatacaagaggtgcttttgctcagcctgcgttctacgaggcttttggacttacggtagtggaagcgatgacttgcgggctcccgacttttgccacttgtcacggtggtccagcagagatcatcgagcacgggctctcgggtttccacatcgatccataccatcctgagcaagcgggtaacataatggctgatttctttgaacgttgtaaggaagatccaaaccattggaagaaagtatcagacgctggtctccaaaggatatacgaaaggtacacatggaagatatactcggagagattgatgacactagctggtgtgtatggtttctggaaatacgtatcgaaattggagcgtcgtgagactcggcgatatcttgaaatgttctacattctcaaattccgcgacttggtgaaaactgttccttcaaccgccgatgactgacccggttcagcgttggatgaagtgttggactgtaaaaaagaataaatgatgagtaactttggctatgtaccctatgttgtgtgtatgtatgaaaggaagaatttgttccatcttccatggagtaattacgaatttggtggtacttttgtgttgtctcatgtgtgtctgactgacatgttgaagattattcacgtgaagtttgtagcttataataaaaagtcttcaatggaacatttcatttcacaaaaaaaaaaaaaaaa

SEQ ID NO: 9 - DNA, 33 bp, synthetic construct
  source 1..33: mol_type = other DNA
ccgtttctggaaattgcgaaacagctggcggat

SEQ ID NO: 10 - DNA, 33 bp, synthetic construct
  source 1..33: mol_type = other DNA
cgcaatttccagaaacgggctgatgtgaccgta

SEQ ID NO: 11 - DNA, 39 bp, synthetic construct
  source 1..39: mol_type = other DNA
agcaccccgattaacctggagagcatcattaagaaaatc

SEQ ID NO: 12 - DNA, 33 bp, synthetic construct
  source 1..33: mol_type = other DNA
gttaatcggggtgctgcacaggtagatcaggaa

SEQ ID NO: 13 - DNA, 33 bp, synthetic construct
  source 1..33: mol_type = other DNA
accctgaaaaaggcgctgaaaatgagcaagccg

SEQ ID NO: 14 - DNA, 33 bp, synthetic construct
  source 1..33: mol_type = other DNA
cgcctttttcagggtcgggttcaggtgcggcgg

SEQ ID NO: 15 - DNA, 33 bp, synthetic construct
  source 1..33: mol_type = other DNA
gcgctggatatgagcaagccgaactttagccgt

SEQ ID NO: 16 - DNA, 33 bp, synthetic construct
  source 1..33: mol_type = other DNA
gctcatatccagcgccttgtgcagggtcgggtt

SEQ ID NO: 17 - DNA, 33 bp, synthetic construct
  source 1..33: mol_type = other DNA
tgggcgccgcacgttgcgaacgaacaaaacatt

SEQ ID NO: 18 - DNA, 33 bp, synthetic construct
  source 1..33: mol_type = other DNA
aacgtgcggcgcccacggctgcagcacgtcgta

SEQ ID NO: 19 - DNA, 33 bp, synthetic construct
  source 1..33: mol_type = other DNA
gcgggtaaatttctgaccagctgcgcggcggtg

SEQ ID NO: 20 - DNA, 33 bp, synthetic construct
  source 1..33: mol_type = other DNA
ggtcagaaatttacccgccggaatgttttgttc

SEQ ID NO: 21 - DNA, 33 bp, synthetic construct
  source 1..33: mol_type = other DNA
ttttttaagaacccgggcgttgagttcccgttt

SEQ ID NO: 22 - DNA, 42 bp, synthetic construct
  source 1..42: mol_type = other DNA
gcccgggttcttaaaaaagctaaagaaatagctgaacaccgc

SEQ ID NO: 23 - DNA, 36 bp, synthetic construct
  source 1..36: mol_type = other DNA
gcggaggaagttgcgaacgaacaaaacattccggcg

SEQ ID NO: 24 - DNA, 36 bp, synthetic construct
  source 1..36: mol_type = other DNA
ttcgttcgcaacttcctccgcccacggctgcagcac

SEQ ID NO: 25 - DNA, 39 bp, synthetic construct
  source 1..39: mol_type = other DNA
ccggaatatgaaaaggttaaaatccgtgagattctggcg

SEQ ID NO: 26 - DNA, 33 bp, synthetic construct
  source 1..33: mol_type = other DNA
cttttcatattccggcaggtggatcgccggaaa

SEQ ID NO: 27 - DNA, 33 bp, synthetic construct
  source 1..33: mol_type = other DNA
ctgatgaaaaccagccgtaccatcgaggcgaaa

SEQ ID NO: 28 - DNA, 33 bp, synthetic construct
  source 1..33: mol_type = other DNA
gctggttttcatcagcatcatctgcttgttacc

SEQ ID NO: 29 - DNA, 36 bp, synthetic construct
  source 1..36: mol_type = other DNA
agccgtgaaatcgaggcgaaatacattgactattgc

SEQ ID NO: 30 - DNA, 30 bp, synthetic construct
  source 1..30: mol_type = other DNA
ctcgatttcacggctggtgcacatcagcat

SEQ ID NO: 31 - DNA, 33 bp, synthetic construct
  source 1..33: mol_type = other DNA
ctgtgcaacaaaaaggtggttccggtgggtccg

SEQ ID NO: 32 - DNA, 33 bp, synthetic construct
  source 1..33: mol_type = other DNA
cacctttttgttgcacagttcggtgcaatagtc

SEQ ID NO: 33 - DNA, 33 bp, synthetic construct
  source 1..33: mol_type = other DNA
ggtccgctgttccaagatctgatcaccaacgat

SEQ ID NO: 34 - DNA, 33 bp, synthetic construct
  source 1..33: mol_type = other DNA
ttggaacagcggacccaccggaaccaccttcca

SEQ ID NO: 35 - DNA, 33 bp, synthetic construct
  source 1..33: mol_type = other DNA
ccgccggttcaagatctgatcaccaacgatgcg

SEQ ID NO: 36 - DNA, 30 bp, synthetic construct
  source 1..30: mol_type = other DNA
atcttgaaccggcggacccaccggaaccac

SEQ ID NO: 37 - DNA, 33 bp, synthetic construct
  source 1..33: mol_type = other DNA
tgggttgttcgttttccgaaaggcgaggaacgt

SEQ ID NO: 38 - DNA, 33 bp, synthetic construct
  source 1..33: mol_type = other DNA
aaaacgaacaacccagatgaagttcacgttgct

SEQ ID NO: 39 - DNA, 33 bp, synthetic construct
  source 1..33: mol_type = other DNA
ggcttcgttagccactgcggttggaacagcgcg

SEQ ID NO: 40 - DNA, 33 bp, synthetic construct
  source 1..33: mol_type = other DNA
gtggctaacgaagccaccggtgctcgggtggtt

SEQ ID NO: 41 - DNA, 41 bp, synthetic construct
  source 1..41: mol_type = other DNA
ccgatccacttcgaccaaccgattaacgcgaaactgatggt

SEQ ID NO: 42 - DNA, 41 bp, synthetic construct
  source 1..41: mol_type = other DNA
cggttggtcgaagtggatcggcatcgcaatgatcggaacgc

SEQ ID NO: 43 - DNA, 30 bp, synthetic construct
  source 1..30: mol_type = other DNA
gcggaagttctgaagagcgtggttaccggc

SEQ ID NO: 44 - DNA, 30 bp, synthetic construct
  source 1..30: mol_type = other DNA
cttcagaacttccgcaatctcgccacggtg

SEQ ID NO: 45 - DNA, 33 bp, synthetic construct
  source 1..33: mol_type = other DNA
aagagcaaacgtgatgaggaaatggacgcggtt

SEQ ID NO: 46 - DNA, 39 bp, synthetic construct
  source 1..39: mol_type = other DNA
ctcatcacgtttgctcttcaggtttttgctgatttcacg

SEQ ID NO: 47 - DNA, 32 bp, synthetic construct
  source 1..32: mol_type = other DNA
aggttttcttgttcccgtggctggcgtatggt

SEQ ID NO: 48 - DNA, 43 bp, synthetic construct
  source 1..43: mol_type = other DNA
cgggaacaagaaaacctttagttttgtgtgttcagtatccata

SEQ ID NO: 49 - DNA, 32 bp, synthetic construct
  source 1..32: mol_type = other DNA
caagaaacgtattccgcaaagctacagcagca

SEQ ID NO: 50 - DNA, 39 bp, synthetic construct
  source 1..39: mol_type = other DNA
gcggaatacgtttcttgatgaagctaaggttgatcggag

SEQ ID NO: 51 - DNA, 32 bp, synthetic construct
  source 1..32: mol_type = other DNA
agcttccgcaactgccaccgcattaccatacc

SEQ ID NO: 52 - DNA, 32 bp, synthetic construct
  source 1..32: mol_type = other DNA
tggcagttgcggaagctccggcaggatcagct

SEQ ID NO: 53 - DNA, 32 bp, synthetic construct
  source 1..32: mol_type = other DNA
gcctcacctgaacagcacgctgcacaaagcgt

SEQ ID NO: 54 - DNA, 32 bp, synthetic construct
  source 1..32: mol_type = other DNA
tgctgttcaggtgaggcggcagaccgttggtg

SEQ ID NO: 55 - DNA, 32 bp, synthetic construct
  source 1..32: mol_type = other DNA
tatgcaaccttggacctttggcgtcgctagtt

SEQ ID NO: 56 - DNA, 35 bp, synthetic construct
  source 1..35: mol_type = other DNA
aggtccaaggttgcataacgtcgtagatgatcaga

SEQ ID NO: 57 - DNA, 32 bp, synthetic construct
  source 1..32: mol_type = other DNA
accctgaagttgagtacccgtttccggcactt

SEQ ID NO: 58 - DNA, 43 bp, synthetic construct
  source 1..43: mol_type = other DNA
gtactcaacttcagggtttttgtagagatgaacgaaatagctg

SEQ ID NO: 59 - DNA, 34 bp, synthetic construct
  source 1..34: mol_type = other DNA
tatggactatttggctgaaatcatcgaaactcgc

SEQ ID NO: 60 - DNA, 37 bp, synthetic construct
  source 1..37: mol_type = other DNA
cagccaaatagtccatatatttgccctccaactcacg

SEQ ID NO: 61 - DNA, 35 bp, synthetic construct
  source 1..35: mol_type = other DNA
tagagattttagtggccctggaggtcgtgcgtgat

SEQ ID NO: 62 - DNA, 35 bp, synthetic construct
  source 1..35: mol_type = other DNA
agggccactaaaatctctaccagcaacttggcgtt

SEQ ID NO: 63 - DNA, 33 bp, synthetic construct
  source 1..33: mol_type = other DNA
gatcgcccgtgtgattaaggacgtgacctctgg

SEQ ID NO: 64 - DNA, 32 bp, synthetic construct
  source 1..32: mol_type = other DNA
taatcacacgggcgatctcttcacggtgcagg

SEQ ID NO: 65 - DNA, 1365 bp, synthetic construct
  source 1..1365: mol_type = other DNA
atggatactgaacacacaaaactaaaggctttcttgttcccgtggctggcgtatggtcatatttccccgtttttggagttggcgaagaaattgtctgatcgtggtttcctgatcgaactgtgttcgactccgatcaaccttagcttcatccagaaacgtattccgcaaagctacagcagcacgatccagctggtggagctgatcctgccggagttcccgcaactgccaccgcattaccataccaccaacggtctgccgctgcacctgaacagcacgctgcacaaagcgttgaagcttgctaagccgaatttgttcaccattctgaaaaccagaaagccggatctgatcatctacgacgttatgcaactgtggacctttggcgtcgctagttcgctcaacatcccgagcgcacgcttctttacctcgggcgcggcaatgtgcagctatttcgttcatctctacaaaaacttggaagttgagtacccgtttccggcacttcacctgtacgactacgaaatcgagcgtgcacgtaaactggtgcagcgtaacgataaagagaatgaaaacaaagacgaccagccagaagaagagatgccgcctcaagaaggtattatgctgattagcacgagccgtgagttggagggcaaatatatgaactatttggctgaaatcatcgaaactcgcatttttccgatcggcactctggtacaggatccggttgccagcggtgacgagaacatgaatattatgcagtggctggacagcaaaaaggaattatctacggtttttgtgtccttcggctctgaatatttcttaaccaaagaggaacgtgaagagatagcgctgggtctggagttgagccaggttaattttatctgggttgttcgtttcccgaaaggcgaaaaacagaatctggaagaggcgctgccacaaggttttttggagcgcgtgggtgaccgcggtatgattgtggagtgggcaccgcaagcgaagatcctgacccacagctccattggcggcttcgtgagccactgcggttggaacagcatctcagaatctattgagtttggcgttccgattattgcgattccgatgcagctggaccaaccgatgaacgccaagttgctggtagagattggtgtggccctggaggtcgtgcgtgatgataatggctccctgcaccgtgaagagatcgcctccgtgattaaggacgtgacctctggggagagcagcgagaccatgcgttgcaaggtgcgcaacctgggtaagaacctgcgcaccaagagcgttgaagatatggatgcgaccgtcgaggaactgcgtgagctggtcggtgaatctagatccaagaacggcagcttttaa

SEQ ID NO: 66 - protein, 454 aa, synthetic construct
MDTEHTKLKAFLFPWLAYGHISPFLELAKKLSDRGFLIELCSTPINLSFIQKRIPQSYSSTIQLVELILPEFPQLPPHYHTTNGLPLHLNSTLHKALKLAKPNLFTILKTRKPDLIIYDVMQLWTFGVASSLNIPSARFFTSGAAMCSYFVHLYKNLEVEYPFPALHLYDYEIERARKLVQRNDKENENKDDQPEEEMPPQEGIMLISTSRELEGKYMNYLAEIIETRIFPIGTLVQDPVASGDENMNIMQWLDSKKELSTVFVSFGSEYFLTKEEREEIALGLELSQVNFIWVVRFPKGEKQNLEEALPQGFLERVGDRGMIVEWAPQAKILTHSSIGGFVSHCGWNSISESIEFGVPIIAIPMQLDQPMNAKLLVEIGVALEVVRDDNGSLHREEIASVIKDVTSGESSETMRCKVRNLGKNLRTKSVEDMDATVEELRELVGESRSKNGSF

SEQ ID NO: 67 - protein, 809 aa, synthetic construct; identical to SEQ ID NO: 7

SEQ ID NO: 68 - DNA, 2904 bp, synthetic construct; identical to SEQ ID NO: 8
  source 1..2904: mol_type = other DNA

SEQ ID NO: 69 - DNA, 1365 bp, synthetic construct; identical to SEQ ID NO: 6
  source 1..1365: mol_type = other DNA